European Patent Application EP 4 711 449 A1, published March 18, 2026. Title: Activation of proliferation of pancreatic islet cells by activation of glucose pathway. Applicant: The University of Tokyo. The sequence listing filed with the application follows.

SEQUENCE LISTING (14 sequences)

SEQ ID NO: 1 - DNA, 1107 bp, Mouse
  source 1..1107: mol_type = genomic DNA
atggacttcgactcgtatcagcactatttctacgactatgactgcggagaggatttctaccgctccacggcgcccagcgaggacatctggaagaaattcgagctggtgccgtcgccccccacgtcgccgccctggggctccggtcccggcgccgtggacccagcctctgggattaatcccggggagccgtggcctggagggggtgccggggacgaggcggaatctcggggccattcgaaagcctggggcaggaattatgcttccatcattcgccgtgactgcatgtggagcggcttctccgcccgagaacggctggagagagtggtgagcgacaggctggccccaggcgcgccccgggggaacccgcccaaagcgcccgctaccccggacggcactcctagtctggaagccagtaacccggcgcccgccacccaatgtcagctgggcgagcccaagactcaggcctgctccgggtccgagagccccagcgattctgaaggtgaagagattgacgtggtgaccgtggagaagaggcgatctctggacatccgaaagccagtcaccatcacggtgcgagcagaccccctggacccctgcatgaagcacttccatatctctatccaccaacagcagcataactatgctgcccgttttcctccagaaagttgctctcaagagggggatcctgagccaggtccccaggaagaggctccggagatagaagctcccaaggagaaagaggaggaggaagaggaagaggaggaagaagagattgtgagccccccacctgtcggaagtgaggctccccagtcctgccaccccaaacctgtcagttctgacactgaggacgtgaccaagaggaagaaccataacttcttggaacgaaaaaggaggaatgacctccgctcccggttcctagccctgcgggaccaggttcccaccctggccagctgctctaaggcccccaaagtcgtgatcctcagcaaggcgttagaatacttgcaggctttggtgggggctgaaaagaaaatggctacagagaaaaggcagctccggtgtcggcaacagcaactgcaaaagagaatcgcgtacctcagtggctactaa

SEQ ID NO: 2 - protein, 368 aa, Mouse
MDFDSYQHYFYDYDCGEDFYRSTAPSEDIWKKFELVPSPPTSPPWGSGPGAVDPASGINPGEPWPGGGAGDEAESRGHSKAWGRNYASIIRRDCMWSGFSARERLERVVSDRLAPGAPRGNPPKAPATPDGTPSLEASNPAPATQCQLGEPKTQACSGSESPSDSEGEEIDVVTVEKRRSLDIRKPVTITVRADPLDPCMKHFHISIHQQQHNYAARFPPESCSQEGDPEPGPQEEAPEIEAPKEKEEEEEEEEEEEIVSPPPVGSEAPQSCHPKPVSSDTEDVTKRKNHNFLERKRRNDLRSRFLALRDQVPTLASCSKAPKVVILSKALEYLQALVGAEKKMATEKRQLRCRQQQLQKRIAYLSGY

SEQ ID NO: 3 - DNA, 1095 bp, Human
  source 1..1095: mol_type = genomic DNA
atggactacgactcgtaccagcactatttctacgactatgactgcggggaggatttctaccgctccacggcgcccagcgaggacatctggaagaaattcgagctggtgccatcgccccccacgtcgccgccctggggcttgggtcccggcgcaggggacccggcccccgggattggtcccccggagccgtggcccggagggtgcaccggagacgaagcggaatcccggggccactcgaaaggctggggcaggaactacgcctccatcatacgccgtgactgcatgtggagcggcttctcggcccgggaacggctggagagagctgtgagcgaccggctcgctcctggcgcgccccgggggaacccgcccaaggcgtccgccgccccggactgcactcccagcctcgaagccggcaacccggcgcccgccgccccctgtccgctgggcgaacccaagacccaggcctgctccgggtccgagagcccaagcgactcggagaatgaagaaattgatgttgtgacagtagagaagaggcagtctctgggtattcggaagccggtcaccatcacggtgcgagcagaccccctggatccctgcatgaagcatttccacatctccatccatcagcaacagcacaactatgctgcccgttttcctccagaaagctgctcccaagaagaggcttcagagaggggtccccaagaagaggttctggagagagatgctgcaggggaaaaggaagatgaggaggatgaagagattgtgagtcccccacctgtagaaagtgaggctgcccagtcctgccaccccaaacctgtcagttctgatactgaggatgtgaccaagaggaagaatcacaacttcctggagcgcaagaggcggaatgacctgcgttcgcgattcttggcgctgagggaccaggtgcccaccctggccagctgctccaaggcccccaaagtagtgatcctaagcaaggccttggaatacttgcaagccctggtgggggctgagaagaggatggctacagagaaaagacagctccgatgccggcagcagcagttgcagaaaagaattgcatacctcactggctactaa

SEQ ID NO: 4 - protein, 364 aa, Human
MDYDSYQHYFYDYDCGEDFYRSTAPSEDIWKKFELVPSPPTSPPWGLGPGAGDPAPGIGPPEPWPGGCTGDEAESRGHSKGWGRNYASIIRRDCMWSGFSARERLERAVSDRLAPGAPRGNPPKASAAPDCTPSLEAGNPAPAAPCPLGEPKTQACSGSESPSDSENEEIDVVTVEKRQSLGIRKPVTITVRADPLDPCMKHFHISIHQQQHNYAARFPPESCSQEEASERGPQEEVLERDAAGEKEDEEDEEIVSPPPVESEAAQSCHPKPVSSDTEDVTKRKNHNFLERKRRNDLRSRFLALRDQVPTLASCSKAPKVVILSKALEYLQALVGAEKRMATEKRQLRCRQQQLQKRIAYLTGY

SEQ ID NO: 5 - DNA, 20 bp, synthetic construct
  misc_feature 1..20: note = Forward primer sequence for amplifying beta-actin gene
  source 1..20: mol_type = other DNA
gccaaccgtgaaaagatgac

SEQ ID NO: 6 - DNA, 19 bp, synthetic construct
  misc_feature 1..19: note = Reverse primer sequence for amplifying beta-actin gene
  source 1..19: mol_type = other DNA
tccggagtccatcacaatg

SEQ ID NO: 7 - DNA, 20 bp, synthetic construct
  misc_feature 1..20: note = Forward primer sequence for amplifying Mycl gene
  source 1..20: mol_type = other DNA
acggcactcctagtctggaa

SEQ ID NO: 8 - DNA, 21 bp, synthetic construct
  misc_feature 1..21: note = Reverse primer sequence for amplifying Mycl gene
  source 1..21: mol_type = other DNA
ccacgtcaatctcttcacctt

SEQ ID NO: 9 - DNA, 19 bp, synthetic construct
  misc_feature 1..19: note = Forward primer sequence for amplifying Fev gene
  source 1..19: mol_type = other DNA
ccgtcggagatggtctttt

SEQ ID NO: 10 - DNA, 20 bp, synthetic construct
  misc_feature 1..20: note = Reverse primer sequence for amplifying Fev gene
  source 1..20: mol_type = other DNA
ccaggagaaactgccacaac

SEQ ID NO: 11 - DNA, 20 bp, synthetic construct
  misc_feature 1..20: note = Forward primer sequence for amplifying Cck gene
  source 1..20: mol_type = other DNA
actgctagcgcgatacatcc

SEQ ID NO: 12 - DNA, 20 bp, synthetic construct
  misc_feature 1..20: note = Reverse primer sequence for amplifying Cck gene
  source 1..20: mol_type = other DNA
tattctatggctggggtcca

SEQ ID NO: 13 - DNA, 20 bp, synthetic construct
  misc_feature 1..20: note = Forward primer sequence for amplifying Pax4 gene
  source 1..20: mol_type = other DNA
gtacttcgggcacttcagga

SEQ ID NO: 14 - DNA, 20 bp, synthetic construct
  misc_feature 1..20: note = Reverse primer sequence for amplifying Pax4 gene
  source 1..20: mol_type = other DNA
ttactgtggggactgggaag